European Patent Specification EP 3 852 617 B1, published September 10, 2025. Title: METHODS OF REVERSING TICAGRELOR ACTIVITY. Applicant: David James Ballance John Lee. The sequence listing filed with the application follows.

SEQUENCE LISTING (86 sequences)

SEQ ID NO: 1 - DNA, 363 bp, Homo sapiens
gaggtgcagctgttggagtctgggggaggcttggtacagcctggggggtccctgagactctcctgtgcagcctctggattcacctttagcagctatgccatgagctgggtccgccaggctccagggaaggggctggagtgggtctcagctattagtggtagtggtggtagcacatactacgcagactccgtgaagggccggttcaccatctccagagacaattccaagaacacgctgtatctgcaaatgaacagcctgagagccgaggacacggccgtgtattactgtgcaacagagtacgacctgcaacggcctttcgggtttgacttctggggcaaggggacaatggtcaccgtctcgagt

SEQ ID NO: 2 - protein, 121 aa, Homo sapiens
EVQLLESGGGLVQPGGSLRLSCAASGFTFSSYAMSWVRQAPGKGLEWVSAISGSGGSTYYADSVKGRFTISRDNSKNTLYLQMNSLRAEDTAVYYCATEYDLQRPFGFDFWGKGTMVTVSS

SEQ ID NO: 3 - protein, 5 aa, Homo sapiens
SYAMS

SEQ ID NO: 4 - protein, 17 aa, Homo sapiens
AISGSGGSTYYADSVKG

SEQ ID NO: 5 - protein, 12 aa, Homo sapiens
EYDLQRPFGFDF

SEQ ID NO: 6 - DNA, 333 bp, Homo sapiens
tcctatgtgctgactcagccaccctcagcgtctggggcccccgggcagagggctaccatctcctgctctggaagcagctccaacatcggaagtaatcttgtgaactggtaccaacaattcccaggagaggcccccaagctcctcatctttagtgacaatcaacgaccctcaggggtccctgaccgattctctggctccaggtctggcacctcagcctccctggccatcagtgggctccagtccgaggatgaggctgattattactgtgcaacgtgggatgacagactggatggttatgtggtattcggcggagggaccaagctgaccgtccta

SEQ ID NO: 7 - protein, 111 aa, Homo sapiens
SYVLTQPPSASGAPGQRATISCSGSSSNIGSNLVNWYQQFPGEAPKLLIFSDNQRPSGVPDRFSGSRSGTSASLAISGLQSEDEADYYCATWDDRLDGYVVFGGGTKLTVL

SEQ ID NO: 8 - protein, 13 aa, Homo sapiens
SGSSSNIGSNLVN

SEQ ID NO: 9 - protein, 7 aa, Homo sapiens
SDNQRPS

SEQ ID NO: 10 - protein, 12 aa, Homo sapiens
ATWDDRLDGYVV

SEQ ID NO: 11 - DNA, 345 bp, Homo sapiens
caggtacagctgcagcagtcaggggctgaggtgaagaagcctggggcctcagtgaaggtttcctgcaaggcttctggatacaccttcattacctatggtattcactgggtgcgccaggcccccggacaagggcttgagtggatgggatggatcgaccccgggcatggttacacaaaatattcacagaagttccagggcagagtcaccattaccagggacacatccgcgagcacagcctacatggagatgagcagcctcagatctgaagacacggctgtgtattactgtgcgagagcggacctgggtgactactggggccggggaaccctggtcaccgtctcgagt

SEQ ID NO: 12 - protein, 115 aa, Homo sapiens
QVQLQQSGAEVKKPGASVKVSCKASGYTFITYGIHWVRQAPGQGLEWMGWIDPGHGYTKYSQKFQGRVTITRDTSASTAYMEMSSLRSEDTAVYYCARADLGDYWGRGTLVTVSS

SEQ ID NO: 13 - protein, 5 aa, Homo sapiens
TYGIH

SEQ ID NO: 14 - protein, 17 aa, Homo sapiens
WIDPGHGYTKYSQKFQG

SEQ ID NO: 15 - protein, 6 aa, Homo sapiens
ADLGDY

SEQ ID NO: 16 - DNA, 330 bp, Homo sapiens
cagtctgtcgtgacgcagccgccctcagtgtctgcggccccaggacagaaggtcaccatctcctgctctggaagcagctccaacattgggaagaattatgtttcctggttccagcagctcccaggtacagcccccaaactcctcatttatgacaatcataagcgaccctcagggattcctgaccgattctctgcctccaagtctggcacgtcagccaccctggtcatctccggtctccagactggggacgaggcccattattactgcggaacatgggataccagactgagtgctggggtgttcggcggagggaccaaggtcaccgtccta

SEQ ID NO: 17 - protein, 110 aa, Homo sapiens
QSVVTQPPSVSAAPGQKVTISCSGSSSNIGKNYVSWFQQLPGTAPKLLIYDNHKRPSGIPDRFSASKSGTSATLVISGLQTGDEAHYYCGTWDTRLSAGVFGGGTKVTVL

SEQ ID NO: 18 - protein, 13 aa, Homo sapiens
SGSSSNIGKNYVS

SEQ ID NO: 19 - protein, 7 aa, Homo sapiens
DNHKRPS

SEQ ID NO: 20 - protein, 11 aa, Homo sapiens
GTWDTRLSAGV

SEQ ID NO: 21 - DNA, 360 bp, Homo sapiens
gaggtgcagctgttggagtctgggggaggcttggtacagcctggggggtccctgagactctcctgtgcagcctctggattcacctttagcagctatgccatgagctgggtccgccaggctccagggaaggggctggagtgggtctcagctattagtggtagtggtggtagcacatactacgcagactccgtgaagggccggttcaccatctccagagacaattccaagaacacgctgtatctgcaaatgaacagcctgagagccgaggacacggccgtgtattactgtggccatgatagtagtggttactcctactcctttgacttctgggggcgggggaccacggtcaccgtctcgagt

SEQ ID NO: 22 - protein, 120 aa, Homo sapiens
EVQLLESGGGLVQPGGSLRLSCAASGFTFSSYAMSWVRQAPGKGLEWVSAISGSGGSTYYADSVKGRFTISRDNSKNTLYLQMNSLRAEDTAVYYCGHDSSGYSYSFDFWGRGTTVTVSS

SEQ ID NO: 23 - protein, 5 aa, Homo sapiens
SYAMS

SEQ ID NO: 24 - protein, 17 aa, Homo sapiens
AISGSGGSTYYADSVKG

SEQ ID NO: 25 - protein, 11 aa, Homo sapiens
DSSGYSYSFDF

SEQ ID NO: 26 - DNA, 330 bp, Homo sapiens
cagtctgtgttgacgcagccgccctcagcgtctgggacccccgggcagagggtcaccatctcttgttctggcaacatctccaacatcggaagtaacactgtcaactggtatcaacacgtcccaggagcggcccccagactcctcatctatgttaatgatcagcggccgtcaggggtccctgaccgattctctggctccaagtctggcacctcagcctccctggccatcagtgggctccagtctgaagatgaggctgattattactgtgcaacgtgggatgacaccctgaatggaggggtcttcggcggagggaccaagctgaccgtccta

SEQ ID NO: 27 - protein, 110 aa, Homo sapiens
QSVLTQPPSASGTPGQRVTISCSGNISNIGSNTVNWYQHVPGAAPRLLIYVNDQRPSGVPDRFSGSKSGTSASLAISGLQSEDEADYYCATWDDTLNGGVFGGGTKLTVL

SEQ ID NO: 28 - protein, 13 aa, Homo sapiens
SGNISNIGSNTVN

SEQ ID NO: 29 - protein, 7 aa, Homo sapiens
VNDQRPS

SEQ ID NO: 30 - protein, 11 aa, Homo sapiens
ATWDDTLNGGV

SEQ ID NO: 31 - DNA, 387 bp, Homo sapiens
caggtgcagctgcaggagtccggggctgaggtgaagaagcctgggtcctcggtgagggtctcctgcaaggcttctggaggcaccttcgacagttatagtatccattgggtgcgccaggcccctggacaagggcttgagtggatgggagggatcatccctgcctttgggacattaagcagcgcacaggacttccaggccagagtcaccattagcgcggacaagtccacgagcacagcctatatggagctgagcggcctgagatctgaggacacggccgtatattactgtgcgagagggtcccatctttacgatttttggagtgcttctcatccccccaatgatgctcttgctatttggggccaaggaaccctggtcaccgtctcgagt

SEQ ID NO: 32 - protein, 129 aa, Homo sapiens
QVQLQESGAEVKKPGSSVRVSCKASGGTFDSYSIHWVRQAPGQGLEWMGGIIPAFGTLSSAQDFQARVTISADKSTSTAYMELSGLRSEDTAVYYCARGSHLYDFWSASHPPNDALAIWGQGTLVTVSS

SEQ ID NO: 33 - protein, 5 aa, Homo sapiens
SYSIH

SEQ ID NO: 34 - protein, 17 aa, Homo sapiens
GIIPAFGTLSSAQDFQA

SEQ ID NO: 35 - protein, 20 aa, Homo sapiens
GSHLYDFWSASHPPNDALAI

SEQ ID NO: 36 - DNA, 330 bp, Homo sapiens
cagtctgtcgtgacgcagccgccctcagtgtctgcggccccaggacagaaggtcaccatctcctgctctggaagcaactccgacattggcaacaattatgtgtcgtggtaccaacagctcccaggaacagcccccaaactcctcatttatgacaataataaacgaccctcagggattcctgaccgattctctggctccaagtctggcacgtcagccaccctggccatcaccggactccaggctggggacgaggccgattattactgcgggacatgggatatcagcctgagcgctggcttgttcggcggagggaccaaggtcaccgtccta

SEQ ID NO: 37 - protein, 110 aa, Homo sapiens
QSVVTQPPSVSAAPGQKVTISCSGSNSDIGNNYVSWYQQLPGTAPKLLIYDNNKRPSGIPDRFSGSKSGTSATLAITGLQAGDEADYYCGTWDISLSAGLFGGGTKVTVL

SEQ ID NO: 38 - protein, 13 aa, Homo sapiens
SGSNSDIGNNYVS

SEQ ID NO: 39 - protein, 7 aa, Homo sapiens
DNNKRPS

SEQ ID NO: 40 - protein, 11 aa, Homo sapiens
GTWDISLSAGL

SEQ ID NO: 41 - DNA, 387 bp, Homo sapiens
caggtgcagctgcaggagtccggggctgaggtgaagaagcctgggtcctcggtgagggtctcctgcaaggcttctggaggcaccttcgacagttatagtatccattgggtgcgccaggcccctggacaagggcttgagtggatgggagggatcatccctgcctttgggacattaagcagcgcacaggacttccaggccagagtcaccattagcgcggacaagtccacgagcacagcctatatggagctgagcggcctgagatctgaggacacggccgtatattactgtgcgagagggagcttcgactacaggttttggagtgcttctcatccccccaatgatgctcttgctatttggggccaaggaaccctggtcaccgtctcgagt

SEQ ID NO: 42 - protein, 129 aa, Homo sapiens
QVQLQESGAEVKKPGSSVRVSCKASGGTFDSYSIHWVRQAPGQGLEWMGGIIPAFGTLSSAQDFQARVTISADKSTSTAYMELSGLRSEDTAVYYCARGSFDYRFWSASHPPNDALAIWGQGTLVTVSS

SEQ ID NO: 43 - protein, 5 aa, Homo sapiens
SYSIH

SEQ ID NO: 44 - protein, 17 aa, Homo sapiens
GIIPAFGTLSSAQDFQA

SEQ ID NO: 45 - protein, 20 aa, Homo sapiens
GSFDYRFWSASHPPNDALAI

SEQ ID NO: 46 - DNA, 330 bp, Homo sapiens; identical to SEQ ID NO: 36

SEQ ID NO: 47 - protein, 110 aa, Homo sapiens; identical to SEQ ID NO: 37

SEQ ID NO: 48 - protein, 13 aa, Homo sapiens
SGSNSDIGNNYVS

SEQ ID NO: 49 - protein, 7 aa, Homo sapiens
DNNKRPS

SEQ ID NO: 50 - protein, 11 aa, Homo sapiens
GTWDISLSAGL

SEQ ID NO: 51 - DNA, 387 bp, Homo sapiens
caggtgcagctgcaggagtccggggctgaggtgaagaagcctgggtcctcggtgagggtctcctgcaaggcttctggaggcaccttcgacagttatagtatccattgggtgcgccaggcccctggacaagggcttgagtggatgggagggatcatccctgcctttgggacattaagcagcgcacaggacttccaggccagagtcaccattagcgcggacaagtccacgagcacagcctatatggagctgagcggcctgagatctgaggacacggccgtatattactgtgcgagaggctccttcgactactacttttggagtgcttctcatccccccaatgatgctcttgctatttggggccaaggaaccctggtcaccgtctcgagt

SEQ ID NO: 52 - protein, 129 aa, Homo sapiens
QVQLQESGAEVKKPGSSVRVSCKASGGTFDSYSIHWVRQAPGQGLEWMGGIIPAFGTLSSAQDFQARVTISADKSTSTAYMELSGLRSEDTAVYYCARGSFDYYFWSASHPPNDALAIWGQGTLVTVSS

SEQ ID NO: 53 - protein, 5 aa, Homo sapiens
SYSIH

SEQ ID NO: 54 - protein, 17 aa, Homo sapiens
GIIPAFGTLSSAQDFQA

SEQ ID NO: 55 - protein, 20 aa, Homo sapiens
GSFDYYFWSASHPPNDALAI

SEQ ID NO: 56 - DNA, 330 bp, Homo sapiens; identical to SEQ ID NO: 36

SEQ ID NO: 57 - protein, 110 aa, Homo sapiens; identical to SEQ ID NO: 37

SEQ ID NO: 58 - protein, 13 aa, Homo sapiens
SGSNSDIGNNYVS

SEQ ID NO: 59 - protein, 7 aa, Homo sapiens
DNNKRPS

SEQ ID NO: 60 - protein, 11 aa, Homo sapiens
GTWDISLSAGL

SEQ ID NO: 61 - DNA, 387 bp, Homo sapiens; identical to SEQ ID NO: 31

SEQ ID NO: 62 - protein, 129 aa, Homo sapiens; identical to SEQ ID NO: 32

SEQ ID NO: 63 - protein, 5 aa, Homo sapiens
SYSIH

SEQ ID NO: 64 - protein, 17 aa, Homo sapiens
GIIPAFGTLSSAQDFQA

SEQ ID NO: 65 - protein, 20 aa, Homo sapiens
GSHLYDFWSASHPPNDALAI

SEQ ID NO: 66 - DNA, 330 bp, Homo sapiens
cagtctgtcgtgacgcagccgccctcagtgtctgcggccccaggacagaaggtcaccatctcctgctctggaagcaactccgacattggcaacaattatgtgtcgtggtaccaacagctcccaggaacagcccccaaactcctcatttatgacaataataaacgaccctcagggattcctgaccgattctctggctccaagtctggcacgtcagccaccctggccatcaccggactccaggctggggacgaggccgattattactgcgggacatggctgtacgaccgggccgtcggcttgttcggcggagggaccaaggtcaccgtccta

SEQ ID NO: 67 - protein, 110 aa, Homo sapiens
QSVVTQPPSVSAAPGQKVTISCSGSNSDIGNNYVSWYQQLPGTAPKLLIYDNNKRPSGIPDRFSGSKSGTSATLAITGLQAGDEADYYCGTWLYDRAVGLFGGGTKVTVL

SEQ ID NO: 68 - protein, 13 aa, Homo sapiens
SGSNSDIGNNYVS

SEQ ID NO: 69 - protein, 7 aa, Homo sapiens
DNNKRPS

SEQ ID NO: 70 - protein, 11 aa, Homo sapiens
GTWLYDRAVGL

SEQ ID NO: 71 - DNA, 387 bp, Homo sapiens; identical to SEQ ID NO: 51

SEQ ID NO: 72 - protein, 129 aa, Homo sapiens; identical to SEQ ID NO: 52

SEQ ID NO: 73 - protein, 5 aa, Homo sapiens
SYSIH

SEQ ID NO: 74 - protein, 17 aa, Homo sapiens
GIIPAFGTLSSAQDFQA

SEQ ID NO: 75 - protein, 20 aa, Homo sapiens
GSFDYYFWSASHPPNDALAI

SEQ ID NO: 76 - DNA, 330 bp, Homo sapiens; identical to SEQ ID NO: 66

SEQ ID NO: 77 - protein, 110 aa, Homo sapiens; identical to SEQ ID NO: 67

SEQ ID NO: 78 - protein, 13 aa, Homo sapiens
SGSNSDIGNNYVS

SEQ ID NO: 79 - protein, 7 aa, Homo sapiens
DNNKRPS

SEQ ID NO: 80 - protein, 11 aa, Homo sapiens
GTWLYDRAVGL

SEQ ID NO: 81 - protein, 234 aa, Homo sapiens
QVQLQESGAEVKKPGSSVRVSCKASGGTFDSYSIHWVRQAPGQGLEWMGGIIPAFGTLSSAQDFQARVTISADKSTSTAYMELSGLRSEDTAVYYCARGSFDYYFWSASHPPNDALAIWGQGTLVTVSSASTKGPSVFPLAPSSKSTSGGTAALGCLVKDYFPEPVTVSWNSGALTSGVHTFPAVLQSSGLYSLSSVVTVPSSSLGTQTYICNVNHKPSNTKVDKRVEPKSCDK

SEQ ID NO: 82 - protein, 216 aa, Homo sapiens
QSVVTQPPSVSAAPGQKVTISCSGSNSDIGNNYVSWYQQLPGTAPKLLIYDNNKRPSGIPDRFSGSKSGTSATLAITGLQAGDEADYYCGTWLYDRAVGLFGGGTKVTVLGQPKAAPSVTLFPPSSEELQANKATLVCLISDFYPGAVTVAWKADSSPVKAGVETTTPSKQSNNKYAASSYLSLTPEQWKSHRSYSCQVTHEGSTVEKTVAPTECS

SEQ ID NO: 83 - protein, 234 aa, Homo sapiens; identical to SEQ ID NO: 81
  PB2452 VH with CH1

SEQ ID NO: 84 - DNA, 702 bp, Homo sapiens
  cDNA encoding PB2452 VH with CH1
caggttcaattgcaagaaagcggtgcagaagttaaaaaaccgggtagcagcgttcgtgttagctgtaaagcaagcggtggcacctttgatagctatagcattcattgggttcgtcaggcaccgggtcagggtctggaatggatgggtggtattattccggcatttggcaccctgagcagcgcacaggattttcaggcacgtgttaccattagcgcagataaaagcaccagcaccgcatatatggaactgagcggtctgcgtagcgaagataccgcagtgtattattgtgcacgtggtagcttcgattattacttttggagcgcaagccatccgcctaatgatgcactggcaatttggggtcagggcaccctggttaccgttagcagcgcaagcaccaaaggtccgagcgtttttccgctggcaccgagcagcaaaagcaccagtggtggcaccgcagcactgggttgtctggttaaagattattttccggaaccggttaccgtgagctggaatagcggtgcactgaccagcggtgttcatacctttccggcagttctgcagagcagcggtctgtatagcctgagcagcgttgttaccgttccgagcagcagcctgggcacccagacctatatttgtaatgttaatcataaaccgagcaataccaaagtggataaacgtgttgaaccgaaaagctgcgataaa

SEQ ID NO: 85 - protein, 216 aa, Homo sapiens; identical to SEQ ID NO: 82
  PB2452 VL with CL

SEQ ID NO: 86 - DNA, 648 bp, Homo sapiens
  cDNA encoding PB2352 VL with CL
cagagcgttgtgacccagcctccgagcgttagcgcagctccgggtcagaaagtgaccattagctgtagcggtagcaatagcgatattggcaataactatgttagctggtatcagcagctgcctggcaccgcaccgaaactgctgatttatgataataacaaacgtccgagcggtattccggatcgttttagcggtagtaaaagcggcaccagcgcaaccctggcaattaccggtctgcaagccggtgatgaagcagattattattgtggcacctggctgtatgatcgtgcagttggtctgtttggtggtggcaccaaagttaccgttctgggtcagccgaaagcagcaccgagcgttaccctgtttccgcctagcagcgaagaactgcaggcaaataaagcaaccctggtttgtctgatcagcgatttttatccgggtgcagttaccgttgcatggaaagcagatagcagtccggttaaagccggtgttgaaaccaccaccccgagcaaacagagcaataacaaatatgcagcaagcagctatctgagcctgacaccggaacagtggaaaagccatcgtagctatagctgtcaggttacccatgaaggtagcaccgttgaaaaaaccgttgcaccgaccgaatgtagc